European Patent Application EP 4 692 127 A1, published February 11, 2026. Title: 一种单链抗体及其体外合成体系和应用. Applicant: 康码（上海）生物科技有限公司. The sequence listing filed with the application follows.

SEQUENCE LISTING (50 sequences)

SEQ ID NO: 1 - protein, 18 aa, synthetic construct
MITETSSPFRSIFSHSGK

SEQ ID NO: 2 - protein, 8 aa, synthetic construct
HHHHHHHH

SEQ ID NO: 3 - protein, 5 aa, synthetic construct
GSGGS

SEQ ID NO: 4 - protein, 214 aa, synthetic construct
DIQMTQSPSSLSASVGDRVTITCRASQDVNTAVAWYQQKPGKAPKLLIYSASFLYSGVPSRFSGSRSGTDFTLTISSLQPEDFATYYCQQHYTTPPTFGQGTKVEIKRTVAAPSVFIFPPSDEQLKSGTASVVCLLNNFYPREAKVQWKVDNALQSGNSQESVTEQDSKDSTYSLSSTLTLSKADYEKHKVYACEVTHQGLSSPVTKSFNRGEC

SEQ ID NO: 5 - protein, 225 aa, synthetic construct
EVQLVESGGGLVQPGGSLRLSCAASGFNIKDTYIHWVRQAPGKGLEWVARIYPTNGYTRYADSVKGRFTISADTSKNTAYLQMNSLRAEDTAVYYCSRWGGDGFYAMDYWGQGTLVTVSSASTKGPSVFPLAPSSKSTSGGTAALGCLVKDYFPEPVTVSWNSGALTSGVHTFPAVLQSSGLYSLSSVVTVPSSSLGTQTYICNVNHKPSNTKVDKKVEPKSCDK

SEQ ID NO: 6 - protein, 450 aa, synthetic construct
EVQLVESGGGLVQPGGSLRLSCAASGFNIKDTYIHWVRQAPGKGLEWVARIYPTNGYTRYADSVKGRFTISADTSKNTAYLQMNSLRAEDTAVYYCSRWGGDGFYAMDYWGQGTLVTVSSASTKGPSVFPLAPSSKSTSGGTAALGCLVKDYFPEPVTVSWNSGALTSGVHTFPAVLQSSGLYSLSSVVTVPSSSLGTQTYICNVNHKPSNTKVDKKVEPKSCDKTHTCPPCPAPELLGGPSVFLFPPKPKDTLMISRTPEVTCVVVDVSHEDPEVKFNWYVDGVEVHNAKTKPREEQYNSTYRVVSVLTVLHQDWLNGKEYKCKVSNKALPAPIEKTISKAKGQPREPQVYTLPPSREEMTKNQVSLTCLVKGFYPSDIAVEWESNGQPENNYKTTPPVLDSDGSFFLYSKLTVDKSRWQQGNVFSCSVMHEALHNHYTQKSLSLSPGK

SEQ ID NO: 7 - protein, 10 aa, synthetic construct
TGGAGTGSGA

SEQ ID NO: 8 - protein, 238 aa, synthetic construct
VSKGEELFTGVVPILVELDGDVNGHKFSVRGEGEGDATNGKLTLKFICTTGKLPVPWPTLVTTLTYGVQCFSRYPDHMKQHDFFKSAMPEGYVQERTISFKDDGTYKTRAEVKFEGDTLVNRIELKGIDFKEDGNILGHKLEYNFNSHNVYITADKQKNGIKANFKIRHNVEDGSVQLADHYQQNTPIGDGPVLLPDNHYLSTQSKLSKDPNEKRDHMVLLEFVTAAGITLGMDELYK

SEQ ID NO: 9 - protein, 6 aa, synthetic construct
SGGGSG

SEQ ID NO: 10 - protein, 15 aa, synthetic construct
GGGGSGGGGSGGGGS

SEQ ID NO: 11 - protein, 25 aa, synthetic construct
GGGGSGGGGSGGGGSGGGGSGGGGS

SEQ ID NO: 12 - protein, 20 aa, synthetic construct
GGGGSGGGGSGGGGSGGGGS

SEQ ID NO: 13 - protein, 20 aa, synthetic construct
GGSGGSGGSGGSGGSGGSGG

SEQ ID NO: 14 - protein, 30 aa, synthetic construct
SGGGSGGGSEGGGSEGGGSEGGGSEGGGSG

SEQ ID NO: 15 - protein, 34 aa, synthetic construct
SGGGSGGGSEGGGSEGGGSEGGGSEGGGSGGGSG

SEQ ID NO: 16 - protein, 34 aa, synthetic construct
RRYEERRYEERRYEERRYEERRYEERRYEERRYE

SEQ ID NO: 17 - protein, 34 aa, synthetic construct
YYEYYYYEYYYYEYYYYEYYYYEYYYYEYYEYYE

SEQ ID NO: 18 - protein, 34 aa, synthetic construct
IKYLEFISEAIIHVLHSRHPGDFGADAQGAMNKA

SEQ ID NO: 19 - protein, 60 aa, synthetic construct
GGSSGSGSGSTGTSSSGTGTSAGTTGTSASTSGSGSGGGGGSGGGGSAGGTATAGASSGS

SEQ ID NO: 20 - protein, 60 aa, synthetic construct
LAQSHATKHKIPIKYLEFISEAIIHVLHSRHPGDFGADAQGAMNKALELFRKDIAAKYKE

SEQ ID NO: 21 - protein, 82 aa, synthetic construct
GGSSGSGSGSTGTSSSGTGTSAGTTGTSASTSGSGSGGGGGSGGGGSAGGTATAGAGSTGGAGSTGGAGSTGGAGTGSGAGS

SEQ ID NO: 22 - protein, 120 aa, synthetic construct
GGSSGSGSGSTGTSSSGTGTSAGTTGTSASTSGSGSGGGGGSGGGGSAGGTATGGSSGGSGGSSGSGSGSTGTSSSGTGTSAGTTGTSASTSGSGSGGGGGSGGGGSAGGTATAGASSGS

SEQ ID NO: 23 - protein, 180 aa, synthetic construct
GGSSGSGSGSTGTSSSGTGTSAGTTGTSASTSGSGSGGGGGSGGGGSAGGTATAGASSGSGGSSGSGSGSTGTSSSGTGTSAGTTGTSASTSGSGSGGGGGSGGGGSAGGTATAGASSGSGGSSGSGSGSTGTSSSGTGTSAGTTGTSASTSGSGSGGGGGSGGGGSAGGTATAGASSGS

SEQ ID NO: 24 - protein, 36 aa, synthetic construct
GSGVPSRFSGSGSGTDFTLTISSLQPEDFATYYSGS

SEQ ID NO: 25 - protein, 36 aa, synthetic construct
GSGEVQLVESGGGLVQPGGSLRLSSAASGFNIKGSG

SEQ ID NO: 26 - protein, 36 aa, synthetic construct
GAGAGSGAGAGSGAGAGSGAGAGSGAGAGSGAGAGS

SEQ ID NO: 27 - protein, 214 aa, synthetic construct
DIVMTQSPDSLAVSLGERATINCKSSESVSNDVAWYQQKPGQPPKLLINYAFHRFTGVPDRFSGSGYGTDFTLTISSLQAEDVAVYYCHQAYSSPYTFGQGTKLEIKRTVAAPSVFIFPPSDEQLKSGTASVVCLLNNFYPREAKVQWKVDNALQSGNSQESVTEQDSKDSTYSLSSTLTLSKADYEKHKVYACEVTHQGLSSPVTKSFNRGEC

SEQ ID NO: 28 - protein, 455 aa, synthetic construct
QVQLQESGPGLVKPSETLSLTCTVSGFSLTSYGVHWIRQPPGKGLEWIGVIYADGSTNYNPSLKSRVTISKDTSKNQVSLKLSSVTAADTAVYYCARAYGNYWYIDVWGQGTTVTVSSASTKGPSVFPLAPCSRSTSESTAALGCLVKDYFPEPVTVSWNSGALTSGVHTFPAVLQSSGLYSLSSVVTVPSSSLGTKTYTCNVDHKPSNTKVDKRVESKYGPPCPPCPAPPVAGGPSVFLFPPKPKDTLMISRTPEVTCVVVAVSQEDPEVQFNWYVDGVEVHNAKTKPREEQFNSTYRVVSVLTVVHQDWLNGKEYKCKVSNKGLPSSIEKTISKAKGQPREPQVYTLPPSQEEMTKNQVSLTCLVKGFYPSDIAVEWESNGQPENNYKTTPPVLDSDGSFFLYSKLTVDKSRWQEGNVFSCSVMHEALHNHYTQKSLSLSLGKTGGAGTGSGA

SEQ ID NO: 29 - protein, 219 aa, synthetic construct
QVQLQESGPGLVKPSETLSLTCTVSGFSLTSYGVHWIRQPPGKGLEWIGVIYADGSTNYNPSLKSRVTISKDTSKNQVSLKLSSVTAADTAVYYCARAYGNYWYIDVWGQGTTVTVSSASTKGPSVFPLAPCSRSTSESTAALGCLVKDYFPEPVTVSWNSGALTSGVHTFPAVLQSSGLYSLSSVVTVPSSSLGTKTYTCNVDHKPSNTKVDKRVESK

SEQ ID NO: 30 - protein, 219 aa, synthetic construct
DIVMTQSPLSLPVTPGEPASISCRSSQSLLYSIGYNYLDWYLQKSGQSPQLLIYLGSNRASGVPDRFSGSGSGTDFTLKISRVEAEDVGFYYCMQALQTPYTFGQGTKLEIKRTVAAPSVFIFPPSDEQLKSGTASVVCLLNNFYPREAKVQWKVDNALQSGNSQESVTEQDSKDSTYSLSSTLTLSKADYEKHKVYACEVTHQGLSSPVTKSFNRGEC

SEQ ID NO: 31 - protein, 451 aa, synthetic construct
EVQLVESGGGLEQPGGSLRLSCAGSGFTFRDYAMTWVRQAPGKGLEWVSSISGSGGNTYYADSVKGRFTISRDNSKNTLYLQMNSLRAEDTAVYYCAKDRLSITIRPRYYGLDVWGQGTTVTVSSASTKGPSVFPLAPCSRSTSESTAALGCLVKDYFPEPVTVSWNSGALTSGVHTFPAVLQSSGLYSLSSVVTVPSSSLGTKTYTCNVDHKPSNTKVDKRVESKYGPPCPPCPAPEFLGGPSVFLFPPKPKDTLMISRTPEVTCVVVDVSQEDPEVQFNWYVDGVEVHNAKTKPREEQFNSTYRVVSVLTVLHQDWLNGKEYKCKVSNKGLPSSIEKTISKAKGQPREPQVYTLPPSQEEMTKNQVSLTCLVKGFYPSDIAVEWESNGQPENNYKTTPPVLDSDGSFFLYSRLTVDKSRWQEGNVFSCSVMHEALHNHYTQKSLSLSLG

SEQ ID NO: 32 - protein, 228 aa, synthetic construct
EVQLVESGGGLEQPGGSLRLSCAGSGFTFRDYAMTWVRQAPGKGLEWVSSISGSGGNTYYADSVKGRFTISRDNSKNTLYLQMNSLRAEDTAVYYCAKDRLSITIRPRYYGLDVWGQGTTVTVSSASTKGPSVFPLAPCSRSTSESTAALGCLVKDYFPEPVTVSWNSGALTSGVHTFPAVLQSSGLYSLSSVVTVPSSSLGTKTYTCNVDHKPSNTKVDKRVESKYG

SEQ ID NO: 33 - protein, 214 aa, synthetic construct
DIQMTQSPSSLSASVGDRVTITCRASQGIRNYLAWYQQKPGKAPKLLIYAASTLQSGVPSRFSGSGSGTDFTLTISSLQPEDVATYYCQRYNRAPYTFGQGTKVEIKRTVAAPSVFIFPPSDEQLKSGTASVVCLLNNFYPREAKVQWKVDNALQSGNSQESVTEQDSKDSTYSLSSTLTLSKADYEKHKVYACEVTHQGLSSPVTKSFNRGEC

SEQ ID NO: 34 - protein, 461 aa, synthetic construct
EVQLVESGGGLVQPGRSLRLSCAASGFTFDDYAMHWVRQAPGKGLEWVSAITWNSGHIDYADSVEGRFTISRDNAKNSLYLQMNSLRAEDTAVYYCAKVSYLSTASSLDYWGQGTLVTVSSASTKGPSVFPLAPSSKSTSGGTAALGCLVKDYFPEPVTVSWNSGALTSGVHTFPAVLQSSGLYSLSSVVTVPSSSLGTQTYICNVNHKPSNTKVDKKVEPKSCDKTHTCPPCPAPELLGGPSVFLFPPKPKDTLMISRTPEVTCVVVDVSHEDPEVKFNWYVDGVEVHNAKTKPREEQYNSTYRVVSVLTVLHQDWLNGKEYKCKVSNKALPAPIEKTISKAKGQPREPQVYTLPPSRDELTKNQVSLTCLVKGFYPSDIAVEWESNGQPENNYKTTPPVLDSDGSFFLYSKLTVDKSRWQQGNVFSCSVMHEALHNHYTQKSLSLSPGKTGGAGTGSGA

SEQ ID NO: 35 - protein, 226 aa, synthetic construct
EVQLVESGGGLVQPGRSLRLSCAASGFTFDDYAMHWVRQAPGKGLEWVSAITWNSGHIDYADSVEGRFTISRDNAKNSLYLQMNSLRAEDTAVYYCAKVSYLSTASSLDYWGQGTLVTVSSASTKGPSVFPLAPSSKSTSGGTAALGCLVKDYFPEPVTVSWNSGALTSGVHTFPAVLQSSGLYSLSSVVTVPSSSLGTQTYICNVNHKPSNTKVDKKVEPKSCDK

SEQ ID NO: 36 - protein, 214 aa, synthetic construct
DIQMTQSPSSLSASVGDRVTITCSASQDISNYLNWYQQKPGKAPKVLIYFTSSLHSGVPSRFSGSGSGTDFTLTISSLQPEDFATYYCQQYSTVPWTFGQGTKVEIKRTVAAPSVFIFPPSDEQLKSGTASVVCLLNNFYPREAKVQWKVDNALQSGNSQESVTEQDSKDSTYSLSSTLTLSKADYEKHKVYACEVTHQGLSSPVTKSFNRGEC

SEQ ID NO: 37 - protein, 463 aa, synthetic construct
EVQLVESGGGLVQPGGSLRLSCAASGYTFTNYGMNWVRQAPGKGLEWVGWINTYTGEPTYAADFKRRFTFSLDTSKSTAYLQMNSLRAEDTAVYYCAKYPHYYGSSHWYFDVWGQGTLVTVSSASTKGPSVFPLAPSSKSTSGGTAALGCLVKDYFPEPVTVSWNSGALTSGVHTFPAVLQSSGLYSLSSVVTVPSSSLGTQTYICNVNHKPSNTKVDKKVEPKSCDKTHTCPPCPAPELLGGPSVFLFPPKPKDTLMISRTPEVTCVVVDVSHEDPEVKFNWYVDGVEVHNAKTKPREEQYNSTYRVVSVLTVLHQDWLNGKEYKCKVSNKALPAPIEKTISKAKGQPREPQVYTLPPSREEMTKNQVSLTCLVKGFYPSDIAVEWESNGQPENNYKTTPPVLDSDGSFFLYSKLTVDKSRWQQGNVFSCSVMHEALHNHYTQKSLSLSPGKTGGAGTGSGA

SEQ ID NO: 38 - protein, 228 aa, synthetic construct
EVQLVESGGGLVQPGGSLRLSCAASGYTFTNYGMNWVRQAPGKGLEWVGWINTYTGEPTYAADFKRRFTFSLDTSKSTAYLQMNSLRAEDTAVYYCAKYPHYYGSSHWYFDVWGQGTLVTVSSASTKGPSVFPLAPSSKSTSGGTAALGCLVKDYFPEPVTVSWNSGALTSGVHTFPAVLQSSGLYSLSSVVTVPSSSLGTQTYICNVNHKPSNTKVDKKVEPKSCDK

SEQ ID NO: 39 - protein, 214 aa, synthetic construct
EIVLTQSPATLSLSPGERATLSCRASQSVSSYLAWYQQKPGQAPRLLIYDASNRATGIPARFSGSGSGTDFTLTISSLEPEDFAVYYCQQRSNWPPTFGQGTKVEIKRTVAAPSVFIFPPSDEQLKSGTASVVCLLNNFYPREAKVQWKVDNALQSGNSQESVTEQDSKDSTYSLSSTLTLSKADYEKHKVYACEVTHQGLSSPVTKSFNRGEC

SEQ ID NO: 40 - protein, 452 aa, synthetic construct
EVQLLESGGGLVQPGGSLRLSCAVSGFTFNSFAMSWVRQAPGKGLEWVSAISGSGGGTYYADSVKGRFTISRDNSKNTLYLQMNSLRAEDTAVYFCAKDKILWFGEPVFDYWGQGTLVTVSSASTKGPSVFPLAPSSKSTSGGTAALGCLVKDYFPEPVTVSWNSGALTSGVHTFPAVLQSSGLYSLSSVVTVPSSSLGTQTYICNVNHKPSNTKVDKRVEPKSCDKTHTCPPCPAPELLGGPSVFLFPPKPKDTLMISRTPEVTCVVVDVSHEDPEVKFNWYVDGVEVHNAKTKPREEQYNSTYRVVSVLTVLHQDWLNGKEYKCKVSNKALPAPIEKTISKAKGQPREPQVYTLPPSREEMTKNQVSLTCLVKGFYPSDIAVEWESNGQPENNYKTTPPVLDSDGSFFLYSKLTVDKSRWQQGNVFSCSVMHEALHNHYTQKSLSLSPGK

SEQ ID NO: 41 - protein, 227 aa, synthetic construct
EVQLLESGGGLVQPGGSLRLSCAVSGFTFNSFAMSWVRQAPGKGLEWVSAISGSGGGTYYADSVKGRFTISRDNSKNTLYLQMNSLRAEDTAVYFCAKDKILWFGEPVFDYWGQGTLVTVSSASTKGPSVFPLAPSSKSTSGGTAALGCLVKDYFPEPVTVSWNSGALTSGVHTFPAVLQSSGLYSLSSVVTVPSSSLGTQTYICNVNHKPSNTKVDKRVEPKSCDK

SEQ ID NO: 42 - protein, 215 aa, synthetic construct
DIQLTQSPSSLSASVGDRVTITCRASQSVDYDGDSYMNWYQQKPGKAPKLLIYAASYLESGVPSRFSGSGSGTDFTLTISSLQPEDFATYYCQQSHEDPYTFGQGTKVEIKRTVAAPSVFIFPPSDEQLKSGTASVVCLLNNFYPREAKVQWKVDNALQSGNSQESVTEQDSKDSTYSLSSTLTLSKADYEKHKVYACEVTHQGLSSPVTKSFNR

SEQ ID NO: 43 - protein, 447 aa, synthetic construct
EVQLVESGGGLVQPGGSLRLSCAVSGYSITSGYSWNWIRQAPGKGLEWVASITYDGSTNYADSVKGRFTISRDDSKNTFYLQMNSLRAEDTAVYYCARGSHYFGHWHFAVWGQGTLVTVSSGPSVFPLAPSSKSTSGGTAALGCLVKDYFPEPVTVSWNSGALTSGVHTFPAVLQSSGLYSLSSVVTVPSSSLGTQTYICNVNHKPSNTKVDKKAEPKSCDKTHTCPPCPAPELLGGPSVFLFPPKPKDTLMISRTPEVTCVVVDVSHEDPEVKFNWYVDGVEVHNAKTKPREEQYNSTYRVVSVLTVLHQDWLNGKEYKCKVSNKALPAPIEKTISKAKGQPREPQVYTLPPSRDELTKNQVSLTCLVKGFYPSDIAVEWESNGQPENNYKTTPPVLDSDGSFFLYSKLTVDKSRWQQGNVFSCSVMHEALHNHYTQKSLSLSPGK

SEQ ID NO: 44 - protein, 222 aa, synthetic construct
EVQLVESGGGLVQPGGSLRLSCAVSGYSITSGYSWNWIRQAPGKGLEWVASITYDGSTNYADSVKGRFTISRDDSKNTFYLQMNSLRAEDTAVYYCARGSHYFGHWHFAVWGQGTLVTVSSGPSVFPLAPSSKSTSGGTAALGCLVKDYFPEPVTVSWNSGALTSGVHTFPAVLQSSGLYSLSSVVTVPSSSLGTQTYICNVNHKPSNTKVDKKAEPKSCDK

SEQ ID NO: 45 - protein, 219 aa, synthetic construct
DVQVTQSPSSLSASVGDRVTITCRSSQSLANSYGNTFLSWYLHKPGKAPQLLIYGISNRFSGVPDRFSGSGSGTDFTLTISSLQPEDFATYYCLQGTHQPYTFGQGTKVEIKRTVAAPSVFIFPPSDEQLKSGTASVVCLLNNFYPREAKVQWKVDNALQSGNSQESVTEQDSKDSTYSLSSTLTLSKADYEKHKVYACEVTHQGLSSPVTKSFNRGEC

SEQ ID NO: 46 - protein, 448 aa, synthetic construct
EVQLVQSGAEVKKPGASVKVSCKASGYRFTNYWIHWVRQAPGQGLEWIGGINPGNNYATYRRKFQGRVTMTADTSTSTVYMELSSLRSEDTAVYYCTREGYGNYGAWFAYWGQGTLVTVSSASTKGPSVFPLAPCSRSTSESTAALGCLVKDYFPEPVTVSWNSGALTSGVHTFPAVLQSSGLYSLSSVVTVPSSSLGTKTYTCNVDHKPSNTKVDKRVESKYGPPCPPCPAPEFLGGPSVFLFPPKPKDTLMISRTPEVTCVVVDVSQEDPEVQFNWYVDGVEVHNAKTKPREEQFNSTYRVVSVLTVLHQDWLNGKEYKCKVSNKGLPSSIEKTISKAKGQPREPQVYTLPPSQEEMTKNQVSLTCLVKGFYPSDIAVEWESNGQPENNYKTTPPVLDSDGSFFLYSRLTVDKSRWQEGNVFSCSVMHEALHNHYTQKSLSLSLGK

SEQ ID NO: 47 - protein, 221 aa, synthetic construct
EVQLVQSGAEVKKPGASVKVSCKASGYRFTNYWIHWVRQAPGQGLEWIGGINPGNNYATYRRKFQGRVTMTADTSTSTVYMELSSLRSEDTAVYYCTREGYGNYGAWFAYWGQGTLVTVSSASTKGPSVFPLAPCSRSTSESTAALGCLVKDYFPEPVTVSWNSGALTSGVHTFPAVLQSSGLYSLSSVVTVPSSSLGTKTYTCNVDHKPSNTKVDKRVES

SEQ ID NO: 48 - protein, 215 aa, synthetic construct
EIVLTQSPGTLSLSPGERATLSCRASQSVRGRYLAWYQQKPGQAPRLLIYGASSRATGIPDRFSGSGSGTDFTLTISRLEPEDFAVFYCQQYGSSPRTFGQGTKVEIKRTVAAPSVFIFPPSDEQLKSGTASVVCLLNNFYPREAKVQWKVDNALQSGNSQESVTEQDSKDSTYSLSSTLTLSKADYEKHKVYACEVTHQGLSSPVTKSFNRGEC

SEQ ID NO: 49 - protein, 452 aa, synthetic construct
EVQLLESGGGLVQPGGSLRLSCAASGFTFSSYAMSWVRQAPGKGLEWVSGITGSGGSTYYADSVKGRFTISRDNSKNTLYLQMNSLRAEDTAVYYCAKDPGTTVIMSWFDPWGQGTLVTVSSASTKGPSVFPLAPSSKSTSGGTAALGCLVKDYFPEPVTVSWNSGALTSGVHTFPAVLQSSGLYSLSSVVTVPSSSLGTQTYICNVNHKPSNTKVDKKVEPKSCDKTHTCPPCPAPELLGGPSVFLFPPKPKDTLMISRTPEVTCVVVDVSHEDPEVKFNWYVDGVEVHNAKTKPREEQYNSTYRVVSVLTVLHQDWLNGKEYKCKVSNKALPAPIEKTISKAKGQPREPQVYTLPPSRDELTKNQVSLTCLVKGFYPSDIAVEWESNGQPENNYKTTPPVLDSDGSFFLYSKLTVDKSRWQQGNVFSCSVMHEALHNHYTQKSLSLSPGK

SEQ ID NO: 50 - protein, 227 aa, synthetic construct
EVQLLESGGGLVQPGGSLRLSCAASGFTFSSYAMSWVRQAPGKGLEWVSGITGSGGSTYYADSVKGRFTISRDNSKNTLYLQMNSLRAEDTAVYYCAKDPGTTVIMSWFDPWGQGTLVTVSSASTKGPSVFPLAPSSKSTSGGTAALGCLVKDYFPEPVTVSWNSGALTSGVHTFPAVLQSSGLYSLSSVVTVPSSSLGTQTYICNVNHKPSNTKVDKKVEPKSCDK